European Patent Specification EP 3 316 676 B1, published August 5, 2026. Title: HAPLOID INDUCER LINE FOR ACCELERATED GENOME EDITING. Applicant: Regents of the University of Minnesota. The sequence listing filed with the application follows.

SEQUENCE LISTING (49 sequences)

SEQ ID NO: 1 - DNA, 4140 bp, Artificial Sequence
  synthetic
atggataagaagtactccatcggactggatatcggaactaactccgtgggatgggctgtgatcactgatgagtacaaggtgccatccaagaagttcaaggtgctgggaaacactgatagacactccatcaagaagaacctgatcggagctctgctgttcgattccggagagactgctgaggctactagactgaagagaactgctagaagaagatacactagaagaaagaacagaatctgctacctgcaagagatcttctccaacgagatggctaaggtggatgattccttcttccacagactggaggagtccttcctggtggaggaggataagaagcacgagagacacccaatcttcggaaacatcgtggatgaggtggcttaccacgagaagtacccaactatctaccacctgagaaagaagctggtggattccactgataaggctgatctgagactgatctacctggctctggctcacatgatcaagttcagaggacacttcctgatcgagggagatctgaacccagataactccgatgtggataagctgttcatccaactggtgcaaacttacaaccaactgttcgaggagaacccaatcaacgcttccggagtggatgctaaggctatcctgtccgctagactgtccaagtccagaagactggagaacctgatcgctcaactgccaggagagaagaagaacggactgttcggaaacctgatcgctctgtccctgggactgactccaaacttcaagtccaacttcgatctggctgaggatgctaagctgcaactgtccaaggatacttacgatgatgatctggataacctgctggctcaaatcggagatcaatacgctgatctgttcctggctgctaagaacctgtccgatgctatcctgctgtccgatatcctgagagtgaacactgagatcactaaggctccactgtccgcttccatgatcaagagatacgatgagcaccaccaagatctgactctgctgaaggctctggtgagacaacaactgccagagaagtacaaggagatcttcttcgatcaatccaagaacggatacgctggatacatcgatggaggagcttcccaagaggagttctacaagttcatcaagccaatcctggagaagatggatggaactgaggagctgctggtgaagctgaacagagaggatctgctgagaaagcaaagaactttcgataacggatccatcccacaccaaatccacctgggagagctgcacgctatcctgagaagacaagaggatttctacccattcctgaaggataacagagagaagatcgagaagatcctgactttcagaatcccatactacgtgggaccactggctagaggaaactccagattcgcttggatgactagaaagtccgaggagactatcactccatggaacttcgaggaggtggtggataagggagcttccgctcaatccttcatcgagagaatgactaacttcgataagaacctgccaaacgagaaggtgctgccaaagcactccctgctgtacgagtacttcactgtgtacaacgagctgactaaggtgaagtacgtgactgagggaatgagaaagccagctttcctgtccggagagcaaaagaaggctatcgtggatctgctgttcaagactaacagaaaggtgactgtgaagcaactgaaggaggattacttcaagaagatcgagtgcttcgattccgtggagatctccggagtggaggatagattcaacgcttccctgggaacttaccacgatctgctgaagatcatcaaggataaggatttcctggataacgaggagaacgaggatatcctggaggatatcgtgctgactctgactctgttcgaggatagagagatgatcgaggagagactgaagacttacgctcacctgttcgatgataaggtgatgaagcaactgaagagaagaagatacactggatggggaagactgtccagaaagctgatcaacggaatcagagataagcaatccggaaagactatcctggatttcctgaagtccgatggattcgctaacagaaacttcatgcaactgatccacgatgattccctgactttcaaggaggatatccaaaaggctcaagtgtccggacaaggagattccctgcacgagcacatcgctaacctggctggatccccagctatcaagaagggaatcctgcaaactgtgaaggtggtggatgagctggtgaaggtgatgggaagacacaagccagagaacatcgtgatcgagatggctagagagaaccaaactactcaaaagggacaaaagaactccagagagagaatgaagagaatcgaggagggaatcaaggagctgggatcccaaatcctgaaggagcacccagtggagaacactcaactgcaaaacgagaagctgtacctgtactacctgcaaaacggaagagatatgtacgtggatcaagagctggatatcaacagactgtccgattacgatgtggatcacatcgtgccacaatccttcctgaaggatgattccatcgataacaaggtgctgactagatccgataagaacagaggaaagtccgataacgtgccatccgaggaggtggtgaagaagatgaagaactactggagacaactgctgaacgctaagctgatcactcaaagaaagttcgataacctgactaaggctgagagaggaggactgtccgagctggataaggctggattcatcaagagacaactggtggagactagacaaatcactaagcacgtggctcaaatcctggattccagaatgaacactaagtacgatgagaacgataagctgatcagagaggtgaaggtgatcactctgaagtccaagctggtgtccgatttcagaaaggatttccaattctacaaggtgagagagatcaacaactaccaccacgctcacgatgcttacctgaacgctgtggtgggaactgctctgatcaagaagtacccaaagctggagtccgagttcgtgtacggagattacaaggtgtacgatgtgagaaagatgatcgctaagtccgagcaagagatcggaaaggctactgctaagtacttcttctactccaacatcatgaacttcttcaagactgagatcactctggctaacggagagatcagaaagagaccactgatcgagactaacggagagactggagagatcgtgtgggataagggaagagatttcgctactgtgagaaaggtgctgtccatgccacaagtgaacatcgtgaagaagactgaggtgcaaactggaggattctccaaggagtccatcctgccaaagagaaactccgataagctgatcgctagaaagaaggattgggatccaaagaagtacggaggattcgattccccaactgtggcttactccgtgctggtggtggctaaggtggagaagggaaagtccaagaagctgaagtccgtgaaggagctgctgggaatcactatcatggagagatcctccttcgagaagaacccaatcgatttcctggaggctaagggatacaaggaggtgaagaaggatctgatcatcaagctgccaaagtactccctgttcgagctggagaacggaagaaagagaatgctggcttccgctggagagctgcaaaagggaaacgagctggctctgccatccaagtacgtgaacttcctgtacctggcttcccactacgagaagctgaagggatccccagaggataacgagcaaaagcaactgttcgtggagcaacacaagcactacctggatgagatcatcgagcaaatctccgagttctccaagagagtgatcctggctgatgctaacctggataaggtgctgtccgcttacaacaagcacagagataagccaatcagagagcaagctgagaacatcatccacctgttcactctgactaacctgggagctccagctgctttcaagtacttcgatactactatcgatagaaagagatacacttccactaaggaggtgctggatgctactctgatccaccaatccatcactggactgtacgagactagaatcgatctgtcccaactgggaggagatctgcaaccaaagaagaagagaaaggtgggaggatga

SEQ ID NO: 2 - protein, 1379 aa, Artificial Sequence
  synthetic
MDKKYSIGLDIGTNSVGWAVITDEYKVPSKKFKVLGNTDRHSIKKNLIGALLFDSGETAEATRLKRTARRRYTRRKNRICYLQEIFSNEMAKVDDSFFHRLEESFLVEEDKKHERHPIFGNIVDEVAYHEKYPTIYHLRKKLVDSTDKADLRLIYLALAHMIKFRGHFLIEGDLNPDNSDVDKLFIQLVQTYNQLFEENPINASGVDAKAILSARLSKSRRLENLIAQLPGEKKNGLFGNLIALSLGLTPNFKSNFDLAEDAKLQLSKDTYDDDLDNLLAQIGDQYADLFLAAKNLSDAILLSDILRVNTEITKAPLSASMIKRYDEHHQDLTLLKALVRQQLPEKYKEIFFDQSKNGYAGYIDGGASQEEFYKFIKPILEKMDGTEELLVKLNREDLLRKQRTFDNGSIPHQIHLGELHAILRRQEDFYPFLKDNREKIEKILTFRIPYYVGPLARGNSRFAWMTRKSEETITPWNFEEVVDKGASAQSFIERMTNFDKNLPNEKVLPKHSLLYEYFTVYNELTKVKYVTEGMRKPAFLSGEQKKAIVDLLFKTNRKVTVKQLKEDYFKKIECFDSVEISGVEDRFNASLGTYHDLLKIIKDKDFLDNEENEDILEDIVLTLTLFEDREMIEERLKTYAHLFDDKVMKQLKRRRYTGWGRLSRKLINGIRDKQSGKTILDFLKSDGFANRNFMQLIHDDSLTFKEDIQKAQVSGQGDSLHEHIANLAGSPAIKKGILQTVKVVDELVKVMGRHKPENIVIEMARENQTTQKGQKNSRERMKRIEEGIKELGSQILKEHPVENTQLQNEKLYLYYLQNGRDMYVDQELDINRLSDYDVDHIVPQSFLKDDSIDNKVLTRSDKNRGKSDNVPSEEVVKKMKNYWRQLLNAKLITQRKFDNLTKAERGGLSELDKAGFIKRQLVETRQITKHVAQILDSRMNTKYDENDKLIREVKVITLKSKLVSDFRKDFQFYKVREINNYHHAHDAYLNAVVGTALIKKYPKLESEFVYGDYKVYDVRKMIAKSEQEIGKATAKYFFYSNIMNFFKTEITLANGEIRKRPLIETNGETGEIVWDKGRDFATVRKVLSMPQVNIVKKTEVQTGGFSKESILPKRNSDKLIARKKDWDPKKYGGFDSPTVAYSVLVVAKVEKGKSKKLKSVKELLGITIMERSSFEKNPIDFLEAKGYKEVKKDLIIKLPKYSLFELENGRKRMLASAGELQKGNELALPSKYVNFLYLASHYEKLKGSPEDNEQKQLFVEQHKHYLDEIIEQISEFSKRVILADANLDKVLSAYNKHRDKPIREQAENIIHLFTLTNLGAPAAFKYFDTTIDRKRYTSTKEVLDATLIHQSITGLYETRIDLSQLGGDLQPKKKRKVGG

SEQ ID NO: 3 - DNA, 36 bp, Artificial Sequence
  synthetic
ctgcaaccaaagaagaagagaaaggtgggaggatga

SEQ ID NO: 4 - protein, 11 aa, Artificial Sequence
  synthetic
LQPKKKRKVGG

SEQ ID NO: 5 - DNA, 571 bp, Artificial Sequence
  synthetic
cggtgaattcaagctttcgttgaacaacggaaactcgacttgccttccgcacaatacatcatttcttcttagctttttttcttcttcttcgttcatacagtttttttttgtttatcagcttacattttcttgaaccgtagctttcgttttcttctttttaactttccattcggagtttttgtatcttgtttcatagtttgtcccaggattagaatgattaggcatcgaaccttcaagaatttgattgaataaaacatcttcattcttaagatatgaagataatcttcaaaaggcccctgggaatctgaaagaagagaagcaggcccatttatatgggaaagaacaatagtatttcttatataggcccatttaagttgaaaacaatcttcaaaagtcccacatcgcttagataagaaaacgaagctgagtttatatacagctagagtcgaagtagtgattgggtcttcgagaagacctgttttagagctagaaatagcaagttaaaataaggctagtccgttatcaacttgaaaaagtggcaccgagtcggtgcttttttttgaattcagcc

SEQ ID NO: 6 - DNA, 30 bp, Artificial Sequence
  synthetic
ccaagcttcccaactacacgatggactcac

SEQ ID NO: 7 - DNA, 34 bp, Artificial Sequence
  synthetic
ccggcgcgccatgtaaagagaagagaggacaaag

SEQ ID NO: 8 - DNA, 30 bp, Artificial Sequence; identical to SEQ ID NO: 6
  synthetic

SEQ ID NO: 9 - DNA, 34 bp, Artificial Sequence; identical to SEQ ID NO: 7
  synthetic

SEQ ID NO: 10 - DNA, 34 bp, Artificial Sequence
  synthetic
cgaaaataaatgaaggcatcaataaaagcttacc

SEQ ID NO: 11 - DNA, 45 bp, Artificial Sequence
  synthetic
gtcagctcggcgcgcctcttcttctcctctgcaatttttcatcac

SEQ ID NO: 12 - DNA, 24 bp, Artificial Sequence
  synthetic
gattgagaatcaagaatacaagaa

SEQ ID NO: 13 - DNA, 24 bp, Artificial Sequence
  synthetic
aaacttcttgtattcttgattctc

SEQ ID NO: 14 - DNA, 24 bp, Artificial Sequence
  synthetic
gattggaaaagttgtagactgaga

SEQ ID NO: 15 - DNA, 24 bp, Artificial Sequence
  synthetic
aaactctcagtctacaacttttcc

SEQ ID NO: 16 - DNA, 23 bp, Artificial Sequence
  synthetic
ggaaaagttgtagactgagatgg

SEQ ID NO: 17 - DNA, 22 bp, Artificial Sequence
  synthetic
gcacgtgtcacgaaaacccatc

SEQ ID NO: 18 - DNA, 24 bp, Artificial Sequence
  synthetic
attgtagtaacataaagttatgta

SEQ ID NO: 19 - DNA, 24 bp, Artificial Sequence
  synthetic
gattgggctccaccgccggcgacg

SEQ ID NO: 20 - DNA, 24 bp, Artificial Sequence
  synthetic
aaaccgtcgccggcggtggagccc

SEQ ID NO: 21 - DNA, 24 bp, Artificial Sequence
  synthetic
gattgaaccaggacaaggtcctca

SEQ ID NO: 22 - DNA, 24 bp, Artificial Sequence
  synthetic
aaactgaggaccttgtcctggttc

SEQ ID NO: 23 - DNA, 23 bp, Artificial Sequence
  synthetic
gggctccaccgccggcgacgtgg

SEQ ID NO: 24 - DNA, 21 bp, Artificial Sequence
  synthetic
cacggtgcttgaattagtgcg

SEQ ID NO: 25 - DNA, 19 bp, Artificial Sequence
  synthetic
ggtcctccatctggcaccg

SEQ ID NO: 26 - DNA, 23 bp, Artificial Sequence
  synthetic
gaaccaggacaaggtcctcatgg

SEQ ID NO: 27 - DNA, 18 bp, Artificial Sequence
  synthetic
ggtggtggacgaggaggc

SEQ ID NO: 28 - DNA, 21 bp, Artificial Sequence
  synthetic
gtagcaccaatgatgagcgag

SEQ ID NO: 29 - DNA, 2499 bp, Zea maize
gtcatggatggagccagtgaactgatgattttttccccaccccgcacgcaacagcatgggtgacaacaaccactcccgctgcggttgggcgagcacatctctacgcacttgacactcacgcaaacctaacgcatactagattaatcatcgccaccaactatcggcgacagaaacgatgggccccgcttctcttaatcacggtgcttgaattagtgcgcgcatagtagtgaaaaataatagtgaaaaataagcagtgcgtgttttggtgtggtggttggtgagccgtccggcccaataaaaacccctcgcaccacctcgtccctcttcgtcgcatcgcacgccatcagcagctagcgcgctcctcgagcccagcagagaaaggccggcctacccactctctctctctctctctccagtctccaccggcagcgctaatcgtaatagccatgggctccaccgccggcgacgtggccgcggtggtggacgaggaggcgtgcatgtacgcgatgcagctggcgtcgtcgtccatcctgcccatgacgctgaagaacgccatcgagctgggcctgctggaggtgctgcagaaggaggccggcggcggcaaggcggcgctggcgcccgaggaggtggtggcgcggatgcccgcggcgcccggcgaccccgccgccgcggcggccatggtggaccgcatgctccgcctgctcgcctcctacgacgtcgtccggtgccagatggaggaccgggacggccggtacgagcgccgctactccgccgcgcccgtctgcaagtggctcacccccaacgaggacggcgtgtccatggccgccctcgcgctcatgaaccaggacaaggtcctcatggagagctggtgagtagtagccgcatcgcatcaaccaccttctacctatctatatccatcacttgttgctgctggcgtgcgcggcatgcatgatgacgagctcgctcatcattggtgctactagtgatttatttcgtccagtaaaattaattaaggtgcgctgctactctactggctgcggctagcacaaggctggaaatagttgttacttgttatacacgatataatatttctctagaacaaaaaagattttttttttataaaaagcaagcaagaaagaaagtgagtgacttcatgtttttcctaaaaaaaagttaggagtgggatggaaaagtcagcaaggaccacttgtttgttgtccactatccatccagtgggtgagacttttttgcgagacggagcactatattattggccgagtcctttttctgtatccgcaaaacggcagccgtcgatcgccggacggatcgacggctcacatgagtgtcgagtccaattccaaccacgagggcggcaaggaaaaccatccgtgctggtctggactttttgccaaactccattcagccattcgccgactgaaggtgaatcttcagacagccagattgtttggtgtctagtgtgtgcgaagatggcgtagaaaagactgagagacagttggctcacacagacaagtgacaactgactatagtatctgcctgcctggctgatgctgatagagatggggactcttgtcctgtctgtttcttgtatgcgctgatctgattctgatcactgccactctgccaggtactatctcaaggacgcggtgctggacggcggcatcccgttcaacaaggcgtacgggatgacggcgttcgagtaccacggcacggactcgcgcttcaaccgcgtgttcaacgagggcatgaagaaccactcggtgatcatcaccaagaagctgctggacttctacacgggcttcgagggcgtgtcgacgctggtggacgtgggcggcggcgtgggcgccacgctgcacgccatcacgtcccgccacccgcacatctccggggtcaacttcgacctgccgcacgtcatctccgaggcgccgccgttccccggcgtgcgccacgtgggcggggacatgttcgcgtccgtgcccgccggcgacgccatcctcatgaagtggatcctccacgactggagcgacgcgcactgcgccacgctgctcaagaactgctacgacgcgctgccggaaaatggcaaggtcatcgtcgtcgagtgcgtgctgccggtcaacacggaggccacccccaaggcgcagggcgtcttccacgtcgacatgatcatgctcgcgcacaaccccggcggcaaggagcggtacgagcgcgagttccgcgagctcgcaaagggcgccggcttctccgggttcaaggccacctacatctacgccaacgcctgggccatcgagttcatcaagtgaaccaccgtcgccgcgatgagatggcatggctgccacatgctttgcttgcttggtcctcgtatcgtacgtcgccgtcgtcgtcttcttctggttattgcgctgctacctcgctgctctcgcgtatgcatgtacttttgcttaattttctttcttcatatcatgcactctggctggcctagac

SEQ ID NO: 30 - DNA, 24 bp, Artificial Sequence
  synthetic
gattgccgctagggcatcttagat

SEQ ID NO: 31 - DNA, 24 bp, Artificial Sequence
  synthetic
aaacatctaagatgccctagcggc

SEQ ID NO: 32 - DNA, 23 bp, Artificial Sequence
  synthetic
gccgctagggcatcttagatagg

SEQ ID NO: 33 - DNA, 23 bp, Artificial Sequence
  synthetic
tgtgcattctttccaaaaggtca

SEQ ID NO: 34 - DNA, 22 bp, Artificial Sequence
  synthetic
gctccaaagggctttagtagga

SEQ ID NO: 35 - DNA, 10581 bp, Triticum turgidum
atgactacaccaatgagtataccgttcgcaactttggaaaagattacaaatgggttctcaaacgatttaataattggaaggggtgggtatggaaacgtttacaaggtatggcttaatacttgatatttccttttttcagcaaatgttcaggctataaacaaataatttaagtgcaataattatgtcaagcaggcagtttacaaaggggaagtgattgctgtgaagttgcttcatgatgatctggtgcaattacttgatgacagacaatttaaaaatgaactttttaaccttttgagggttgagcatccgaatattgtttgcttacgtggttattgttatgaaacacggtataaaattgttaagcacaatggtgagacagtctttggtaaacatatacacagagttctctgctttgaatacttggagggtggaagcctagacaatcatcttcatggtacgatggaacttcaaaatacagttattttgttttacgtttaaaggaaactgatttctcatttacatacatactctttgttaacttgcgtagcaccatctttgccacctaactggaccacacgttacaataccataaaggggatttgtgaaggcttaaatttccttcacggatgtcaaccaccaattttgcatcttgatctgaagcctgccaatatattagtagacagttccatggtgcctaaactggcggattttggattgtcaaagctcttccatggatcacatactcatgtgacaaaacaaatcataggaacccagtaagcggaagcgacccgtggattgtctcgttctgaattttctttcttttgtgatcaaataaatagtatgtacagttctgtactaactgtgtctttgtatcacgcaggaagtacatgccaccggaattcatcaaagatggcaagatctcggttaaaaatgatgtctttagtttgggtattgtgatcatagaaataatggcaggacctatgggttattcagaattttcagaaatgggcagcggtgcacaatttgtgaaggaggtaataaaaaaaactcaagtttgacacccgagttcgtataaataacaaactaccacaccaagaatttgatgtctaatgtgtgagccattataatcgttgaactgagtttatgacaggaccggcagtaataaaaaatatagcaacactcccccacacaatatattgagcatagaagatacaacttatctagctataacaaaataataatccagaaaagtagccatttttttttccggacaggattgaggtccaccagtccaataactatgaagcagctcgctgatagaaaattccaaggtacaattatttttgtaagtttctccttatcacgtgtgaaacaccaatgtaataaagctgataaaccaaacgtacccactatgagaactgcatacactgagactcgaagaaaagaacaaatgcatatctagaaccttgctccatgggatatctagaaccttgctccatgggatctagcaccatctccattttggagcaagcacgaggtgcgtatcgtaatctttttctgctagatgcagacttagacacccagtattctctaggtaaattatttatctggaaagtcgtaggtaacacttgtgaacaaggatatagcgtacatatatatgggagcatttgtgttatgtgacacttttgacttaattgcaaatattatgttatgtgaagactcaagagtgtttttgaacaagtatcgtacatattgtaccgaaaaaggctttcgccccgctttatattataaagcacatgcccaagccaacaaaccacacaggttcacaaacacacgcagacccacacacaccaagttcacacacagacaagatccacaagggttaatgctgagggcacagcttaacaagccctagaacaaaaaggaaagacaccatctagtcgggctccggggggggggggggggggggcggcggaagtggaggcgccaggcggaaggcgagcgatcgaaggtcggcgaggagggtgttgatgatgtcccgatcctgagggcggctaagcggccgccaaagctgcaagtacccacacattttaaaaatggcgtcagtagcgcgtcgtagagggactttttggatgacaagcttattgcggacggtccacagcgtccagccgagaaccccaacgcataaccaacggatatgtcggtggcgtggggggggaggcgtggatttccgcgaggaggtcggggaagttggagttgcaccactatccgccaaccgtctcacggaaactggaccaaagaaactggccgcagggcacgtgaagaagatgtggttagcatcctccgcagtgccgcacaaggggcaaagcccatccccgggtccgttgcgcttgaggacttcgacaccggaggggaggcggccacgaatccactgccaaaggaagatcctaatcttcagaggtaagcgaatgtcccagatcagagcaaagggctcgggcgcgggcgaaggcgcaatagccgcgtacatgacctagtagagaaacgaccggaggactctaggcgccacgagatggcgtccggggcgtcggtgacgctcatcggaagaagggcgatgtcctggaggagggaatcccaggcggccacttcggggggaccgaaaggacgacgaaacgcgaggcgccctaagtcaataagggccgtctcgacagagacccgagggtcaaccgcaatggtgaagagatcgggaaagcgggcggccagaggggtgtcaccgagccaccgatcaaaccagaacagggtcgcggacccagtaccaatcgaaatggacgtgccgatacgaagcacaggaagcagccgcacgacggcctgccaaaactgtgatccgcccgaacgctgacagaaagccagaggctggccacggaggtatttgttgcggataatggtgagccacaaccctccgtcaccattggcaatacgccacaaccaccgggtcaggagggcgatgttcattcggcgggaggacagaatctcaagacccccctggtctttaggtttacaaatgtccggccaagtcaccatgtggtacttctgtttgtcatcgtcgccagcccaatagaacctggattggtacttggcaatttccgtgtgcagcgtttcatggaggctataaaagctcatgaggaaccaaaggagactggcgagtgaggagttgatgaggatcacccgcgccgcctttgatagccaacgccctttccaaggttcgacgcggtgttgcatacgggtcaccgtagggtggaggtccgccacggtgaggcgcgagtcactaacggggatccccaggtaggtcgtggggaaggaccctagccgacagttcaggcgatcagcaatatcctgagcctcctccggagggtatccaaggaccatcacctcgctcttatcaaagttaatcgtaaggcccgacatctgctggaagcacaggaggaggaacttcaggttagcaacatcctgatttgaaccttccaccattattatggtgtcgttcgcgtattgcaggagggagacccctccccctccaactaggtgagggacaatgccgtggatatggccagcacccttagccttatccaggatggcggccagagcatcgaccaccatgttgaacaggaacggcgagaatgggtctcctgacagaccccacagagggtggggaagtatggcccaatctcgccgttaatgttcaccgccgtctttccacatgaaactgattgcatcacgcgggtcacccagcggtcatcaaagcccttacgcagcagtacttcccgaaggaagggccagtgaacagtatcataggctttatggaagtcaagcttcaggaacacagcacgaagatgcttcacccggacctcgtgaaggacttcatggaataccaacacgccatcaagaataaaccggccttggatgaaggccgattggttcgggtgagtgatcgaatcagccagcagggtcaccctattggcgtaccctttggccaggatccgaaaaatcacgttaatcaccgtgatggggcggaactggcgaatatcagaggcacccggaacctttgggatgagggtaatgatcccatagttgaggcgtcccaggtccatcgaacccgaatagaactcctcgaacaaagccatgacctccggtttgaccgcctgccagaatgttttaaagaaagcaacaggcaggccatccgggcctggggccgaggcggggttcatgcctttaatggccgcgagcacctcgtcctcggcgaagggagcaaccagggccgcattggcctcgccgggaaccaactgcgcccccgtccaagtatcgggggcatcgtacatattgttatatgctccatctctaattgtatctctatatttcggttttgtaggtacttaccaattggagtactatcattaaagctacatcagagtatccagcagaggaactacatcaagtgaatttgtgcatcgacatagcaatgctttgtgtggattctgaaagagtcaatagacccaccatagctggtatcctagatgcattgaataggacaaaaactcatatgccctcctctacgaaaaaaactcatattccctggggacaggtatgatttgcatacttgcaaacaaaatgaaatctcgagtatatatttgcaatctgtagaagacagttgcttggatatatggaccactaagtagttatagagtttgcagctccccgtctcccactcattttattctcaatcaagtagttctttaatagtcaggaacttgcttactgcatccttttgactccctgctctataatccatgtagaagaaccttcattttagttccggctaattccaggaatagaaaactagagagggcctattcgtaatcgtgccttccggagtgacaggctaagtgaagggcagggggatgctgccctcgacaaccgtggctgtgattggcactgtcgtgctcatacgaggtaccagacggtgtagaagttaacctagttgattaatcttaggtgtggtcatgctagatagctatatgaaagagccatacatgtagttcaagtagtgcatgcaagattccaacattcaaaatcgtgccttgtactatggaaggggaaagggaggggtaacacgtaatgagtgccctataagccttacacaatagctttatcagaccactgtggcgccctaactgacgccaacagaggtagctgcaatggttcgatgagatagcggtgagagagaaggggcagggggacattggtggcaggtgtaagggaaaaagggagaggagtgaagccggctgggtaccttggtgggggagaggaaagggtggaggaagaacaaagaggtgaggcgcctgctagtgattgcactgtaagcctaccgcgcgacattgctccaaagctacgctctcccaataaaggagaacttctagagagttgatatgaattaaagagattaccacagactcacatagtgcctgaggtattagccacatttcctttcatgcccttgccgaggggctttcctcggcgcctctcactttgggctttgcttcttcaaaggtggtgtttaggccgcaaagagtacaaccagtgtgttatgtgtgtgcactttcggtgtgttacaatttgccattattgcttgatgctttattactattcaaaatagtttctctttttccaagttgtcattttaacatagcattatagattttgtccttccgatttgcatgttttgatcgtctataacttagtttacataatggaagcacatcccagagagtaaattgatcatgagatcttgaccatgatgattctcctgtttttttccttgtacttacacataaaagttgtttcagttggaagatgtgcccctgtgttcgacaattggtcccaaaagtacgagtaaaaggtcgaacccagttcccacaaaggaaaataaaaggttgaagatgatgacaactgaagtggacaatatcgcgaacaaacaccaacagtttaattgcatgccaggagatagctctaaaactattgttcagcaagttccagacagggaaacatcatcagatgtggaaccgacattaatcattggaagggatgaagaaaaacataaaatattgtccattttatctgagagcaacgcagaagagatgaccatccttccaatatatggcatcggaggaattggcaagacaaccttggcacaattggtgttcaatgacatacagttccgggactactatcgggtgtgggtatatgtttctcagaagtttgacttaaagaaaattggcaactttataatatcacagttaacaaaagagaccagcgatatagatgaccagcagacacttcataatcgccttagacagctatttgctggtaagagtatccttattgttttagatgacctgtgggaggagaaacaacatgagttagagaaattgaaggctatgctaaggcttggcataggaaacaaggttgtcatagtaactacacgtgatgaagccattgcaaggaaaatcaacaggactgttatgccatacaagctagagattttaacagatgatatgtgctggtctataataaaacaaaaaagtttctttgaagatcgatgtgacaaagaacaattggggcagatcggaatggacattgcaatcaagtgtggaggtgtggctttggcggctcaatcacttgggtacatgttgagggagatggagtctgaccaatgggagtcagtgagggacagttatatctggaatctatctactatggaagatccatcattaagaaatcatgaagtgcttctgtccttgctgttaagctattcccatatgcatgaattcttgcagttatgcttttcctattgtgcattctttccaaaaggtcaaaatatagtgaagtatgatctaattcaccagtggatagctcttggattcaccggtccatctggaatatttgattctattcagctctgtgagaaatatattacacggcttttggggatgtcattccttcaatattcaaagacacgttcggtgagttactacatactctcgatgtcccaaaagatagctatgggtagtttcttcatgtcaaagagtccccttccagtactgctaggtgtcaggtttctagaaggccgctagggcatcttagatagggtcatagttatacactactcatcctcaaatgcatatgcctgtgcaattttcttttctagatgaccttctcgacaagctcgttgacatttatcctttttctttttcttttctttcccttgttttcaaccttacctttcaaatttccttttccaagaatgacattcaagtccataacctgatcgtggatatgggtcctactaaagccctttggagctcaatatttttcaactatttcattaaaatgaattcacatctataatcatcatttcttttgttatgtatgtatataaaacaatactaattattgttgaactaataaacacatcgttgattacctctaaacaaatttgaatgtcattaaatttgtcttcatattttttagtgggataagaccccaatccaacaggcgcccaaacaaatggacctatgtactgaaacgttgctgttgctggtgcatttgtagtgctgggtattaattttagcaggtttaagatgaaaaccactgcagatatttatcccaggcattatttcatttgatataagctttgaagtttacagatccatagtgtaatctactctggtgtaatttaaatatactgatccgttgcccattatcgagaaaacatacagctacggttacactcttttatagtgatacaaaagtatttctgttgataaaatatactactataaaacaaaataaattcaatattctaacaacattacgtggttttgctgcagagtgatgaacggcaggacaaagatgttaaaatgtttgtaatgcatgacctagtgcacgatcttgcaagagcaatattggctgataaagttaataaagagggtgatgctgtgggaagcagttgtcactatgcattgctcacagattgtagcaagccattgcagttgtctgttagttcaactgaatatagccggttcaatttttttcttagcctgtttaaaaagaagagttcacatgaaaatataaaggcgttacgttttctgaactgtggcaaagtactacttcgcggtgatgcattttcacctgccaagttcctccttgtcttagatctaagtgaatgctttattcagaagctctcacttgattcgattggacaactgaggcacttgagatatctttgtgctccacgggtcaacgattacacgattcccaactgtatcaccaagctctcagaattaacttacctcaaccttagaggctcttgtcgtatctcagcattgccagagtcaattggcgatatgaaaagtctgatgcatcttgatttatcaggctgctgtgacataattgaactcccagtatcatttgcgaagctgaaacagttggtgcatctagatttatcacactgtcacgtgtctgtatcagaagattttggtggctttaccaaacttcaatatttgaatttatcagttttgtttagttcttccaaggggcataggagaggactgctagaggtcattggcaatttaaagaaactcaggtatctaaatctatctcggtgcatggaggacatagccacatcagaaaaccaaattggcagtttgcttgactctatcagtaccctttccaaccttgagcatctggacttgtctgagaataaacagctttccagtataccagaaagtatgggcaacctcaggaagcttcatacattggacctcttaggctgctatcaactagagaagcttcctgatagtatgattaatatggttagcctgaaggttctaaatgtgggtaatttggttacactggatgaatctgtgctctctttgttaaatattgcctccttgccacactttgtggtgcatgcttcaagtggtaaatgtagcagcaatatcacccgtcttcaggctacaaatcctgatagactgattatagatagacttgaaaatgtcaaatctgcagaagaggcacataacataaaactgatagagaaacagaaaattgaaaccctacaatttgaatggactgtggctgctaggaggtttgtggatgacaaagaggtgttggaaaaactagtgccgccaagcagtgtcgacagtttgtgtataattggttatagaagtgtcagcattcctgattggcttctgggtattagtcagtatctccctaatcttgcgattataagtctggttaatttttctaagtgcaagaacctaccaccactcggtcaactaccaaacttacaatggctgactctcagcagtatggatggtttggaggagtggaacacgacatatactactggagagcaaggtagaaacgaactcttgttccctaagcttgagagattaaacatacatgactgtgccaagttgaggatagaaccatgtctgcctagagctttgtatttgcgcatacgagatagtaataatgtgctatcctcactcaatacaagagagcaagctgagagcacgctgccctcggacatagcacattgtgataatatgatatcagcatgcggaaagagttcgtcatacagcggtgcttcctcttcttctccaataactgatctgtttgtagaggaaagcaaactacccttgcatcagtggaggttgcttcaccaactccccgcgctccgtggtttacggatcaaacattgcagtgatctgaccacctcacttgctgttatccaaaaactctcctccctccaaaatttgagcctggagctcaacgaccatgaactgccgagttggttgattcagctgacagatctacaggaattaaagcttatgcattgcaatagcattacatcactaccacagtggtttggagaacttgcatctctcaagagaattgagatcaagtactgcaaggggatcagctctttgccggagagcatacaacaactgactaagcttgaatttctaagcattcatggctgtcctgtattagaggagtggtgtgaatcagaggagaacaagatgaagctcactcacatcaaagttgaggtatgtgcgtgcaagttatctgttgtattgcttttattctcgtgctggtagtgacttaatactcttttcttaaatggcaagtatacacatgccatgagtatctttacataatcatggtaagtgttgaattaggtgtatgtattttgtctattagatgcttcatgtgtctagattacttgacaaaaatatgtgacgactgcattaataattcgcctaagaagaaaagcattccagttgtgattgtgctatatcatgcacctatacatgcattgttctgattatatatcccgtttgcattgttcagatcgctggacgggattcggtaggctttgaggattcgaaggttcagattgtcaaaccaatgccagcacaaatggttcgccaatcagcatttgctactacagaacgaagatag

SEQ ID NO: 36 - DNA, 24 bp, Artificial Sequence
  synthetic
gattgggtgccggtggcaggatga

SEQ ID NO: 37 - DNA, 24 bp, Artificial Sequence
  synthetic
aaactcatcctgccaccggcaccc

SEQ ID NO: 38 - DNA, 23 bp, Artificial Sequence
  synthetic
gggtgccggtggcaggatgacgg

SEQ ID NO: 39 - DNA, 20 bp, Artificial Sequence
  synthetic
ttcgtcccgtcaacaagagg

SEQ ID NO: 40 - DNA, 19 bp, Artificial Sequence
  synthetic
gtccgtcggcgagcgctgg

SEQ ID NO: 41 - DNA, 1553 bp, Avena sativa
cataaaccactcgttcgtcccgtcaacaagaggagcagaggcgagggactcgcgctcgcgtgtgtggtgtccttccctcgatctgcccctctccggccagttctatcacctcctatcagcaacatgggtgccggtggcaggatgacggagaaggagagggagaagcaggagcagctcggccgcgccgacgtcggtgcgaccctccagcgctcgccgacggacaagccgccgttcacactggggcagatcaagaaggcgatcccaccccactgcttccagcgctcggtgatcaagtcattctcctacgtggtccatgacctcgtcatcgtggctgctctcctgtacgccgcgctggtctggatccccaccctcccgagcgtgctgcagctgggcgcctggccgctctactggatcgtgcagggctgcgtcatgaccggcgtctgggtcatcgcgcacgagtgcggccaccacgccttctccgactactcgctcctcgacgacatcgtcggcctggtgctccactcgtggctgctggtcccgtacttctcgtggaagtacagccaccgtcgccaccactccaacaccggctccatggagcgtgacgaggtgttcgtccccaagcagaaggacgcgctggcctggtacaccccatacatctacaacaaccccatcggccgtctggtgcacatcgtggtgcagctcaccctcgggtggccgctgtacctgtcgatgaacgcctcgggccgcccgtacgcgcgcttcgcctgccacttcgacccctacggccccatctacaacgaccgggagcgcgtccagatcttcatttcggacgtcggtgtggtggccacggcgttcaccctcttcaagcttgcttcggcgttcgggttctggtgggtggtgcgcatctacggtgtgccgctgctgatcgtgaacgcgtggctggtcctgatcacctacctgcagcacacccacccggcgctgccgcactacgactccaccgagtgggactggctgcggggggcgctggccaccatggaccgggactacggcatcctcaaccgcgtgttccacaacatcacggacacgcacgtggcgcaccacctcttctccaccatgccgcactaccatgccatggaggccaccaaggcgatcaagccaatcctgggcgagtactaccagttcgaccccacccccgtggccaaggcaacatggcgcgaggccaaggagtgcatctacgtcgcgcccaccgaggaccgcaagggcgtcttctggtacagcaacaagttctagattcgtcatggggacctgctgtgctgctggaatgtgaggaggaagaagtcagtaatacaccaagtatccatccatctacctacatatggttgggggttagtagtctttagatagaagagagcgttgtttgggcacaaggaaaagactatgaccaccgtgccaatgctagaagagtcgaagcaggtgcaacgaggagtagcgtgtcgggtgtccgtggctttggtcagttccgtcctgtgtctttacttcctagtcgccggttt

SEQ ID NO: 42 - DNA, 24 bp, Artificial Sequence
  synthetic
gattggcggaggggatggtgacgg

SEQ ID NO: 43 - DNA, 24 bp, Artificial Sequence
  synthetic
aaacccgtcaccatcccctccgcc

SEQ ID NO: 44 - DNA, 23 bp, Artificial Sequence
  synthetic
ggcggaggggatggtgacggtgg

SEQ ID NO: 45 - DNA, 20 bp, Artificial Sequence
  synthetic
tccaacgtggacacgacttt

SEQ ID NO: 46 - DNA, 20 bp, Artificial Sequence
  synthetic
gaggtggcatttgtggagga

SEQ ID NO: 47 - DNA, 2147 bp, Hordeum vulgare
gtcataactcggcaaacatagattagacagaattttctgagttcttatctagaggaactcgatgaacttgaggcattgtcgaggttcttcctttcaccgagtacttttttgcgtgtactaggcaaatatatgaagtttgtgagtttcggatcaccaccgagtgcaagtttggaccaaacttgacaaatacataagtttggcgagctccgaatgaaatgaactctgcaaaagaatagaactcggcgcaaaaccagattctaatagtgtgtgaatttttgggctgttttgtataaatatgatgaaacttagtaaaatttcactcaggtcaatgctaatgtggagagtaaataaaaaatgaagggagtacttggctgcatcatatgtttgcccccgatcaccttcacatctccccgtccggacggcctggatcggaaagcactcagccggagccccgccggcgcttgccgttgggtacctctgccacctatttatattacccctaggtctctccctggagacacgcactcccctccttcaactagtgctttgcggcccgtggtcctcctctcgatccagttcctgagcacaccaacaggcaacagaacaacctaccgtgtctcccctccaatctcctcacgatcccttctttccctcagatccgaaccgaaagcatggacaagcatcagctctttgattcatccaacgtggacacgactttcttcgcggccaatggtacacacgacgccgcgcgcgcccggtctttgcgcatgcgatgatgcagctgcagtagcttcagtttcaccggccaggacacgcatgtgatgacgttttttccattctgtgtttgtatgtgcaggcacggcgcagggggataccagcaagcagagggcgcggcgcaggcggcggaggtcggcgaggtgcggcggaggggatggtgacggtggggagatggacggaggaggggaccccaagaagcggcggctcaccgacgagcaggccgagattctggagctgagcttccgggaggaccgcaagctggagacagcccgcaaggtgtatctggccgccgagctcgggctggaccccaagcaggtcgccgtgtggttccagaaccgccgcgcgcgccacaagaacaagacgctcgaggaggagttcgcgaggctcaagcacgcccacgacgccgccatcctccacaaatgccacctcgagaacgaggtatgcttgctcgcatacactcacactggcttacatatggcgctgcacatctgcagttcctctccgttcttgaacatgcttactgacaaacatatggccagctgctgaggctgaaggagagactgggagcgactgagcaggaggtgcggcgcctcaggtcggcagctgggagccacggggcatctgtggatggcggacacgccgctggcgccgttggcgtgtgcggcgggagcccgagctcgtccttctcgacgggaacctgccagcagcagccgggtttcagcggggcagacgtgctggggcgggacgatgacctgatgatgtgcgtccccgagtggtttttagcatgaattagagtttatgctggctaagccgatagcagcgtggtcgagtgttttttagcatgaaatcagatctccatctcccataaaatagccgagatagctgctgccgccgccaaatcctctatagggcttcaagatcggcagaaacctctagaaatcatctcccccctccggaaaagtcgcctctatttgtctccattgcccgcgatgcagcatccggtatagctgctaagacaggccgcccctaaatcgtttctccagcgattttaatctttggtttttagcctgtatatatgggctgtgatttgaagttgagacgagctggacatcaactgcacgctgatcgattactattctagtttggcatagtgttaattaagtttggatgatctctaggcgtgcgttaagtatgtagatagtgttgattaatggcaaaagcttgcaagttaagtgtagtattggcagctctcttgaagatcaaatatgatgtgtgttatcatttgatgatatatattttacttcagccgtaaatagtcttcttagggaagcactgtccatgtatgtgctggtagttggcattcatctttc

SEQ ID NO: 48 - protein, 9 aa, Artificial Sequence
  consensus
LAGLIDADG

SEQ ID NO: 49 - protein, 13 aa, Artificial Sequence
  mutant
GGGCCCGGCGACG